European Patent Specification EP 3 576 785 B1, published February 19, 2025. Title: Virus-Like Particle. Applicant: Pharmaq AS NILSEN, Pal RODE, Marit. The sequence listing filed with the application follows.

SEQUENCE LISTING (2 sequences)

SEQ ID NO: 1 - DNA, 2586 bp, Piscine Myocarditis Virus
atggaaccaaacacatctgtcattgcaacggagcagcagcaggctgccatgagagaggtggaggccgaggcggcggccagagacgaagtggtggagaagatcgcattcgctgaaggagcgatgatggtacagacgaggaggttaccatcaggaaagtcgtcggtaggaggttttctcggcgaactggcacagaacatacgtgccatgaatcggtcattgcacacagataccaacatgctgaccgaaggggcgatggtggacagagcgagggcaaaagtacacaaaatcattagggaagggaatttggactctagggtattttcaaacacggggagcaacactatgttgtcactgtgggtaccagcagtaccgggaccaccggcagtaccggagcattgggacgttgcgccgtcctggttcgtatgcagaccggggaaaaagggggggataaagatcacacaaagcgcatcaatggcagcattaaacccactatttagaggcgcagacgtggggccaatcgggacagcagtcagggcggatgtaaacgcattttcaatgaatgcagttctgggagcactaagagccgggggatttaacaccgaacattccctggtgtcattcgttgaaccactaattcggatcttgctaatgggggtacaaacacaagacagggggaccagcccatgggattgggttggagggatgagttcgcgaatagtcaatcccctagtattcacaacaagcgggaacttcttcccagggggaccaaatttgagggtgtggggagccaacgatacagtggccaggatagtaaacgttgaggactacatgcgcgaggcggccggggaggggaggttcgacgctggatggggaccggaattctggggtgggacaggggacgacgcagtggcggtggtaccgataagggcagtagaagcagggctaggagaagtaaacgcagggtggacattggcacacatggaatacccagtcaaggttagactacttgacgtcgacgaccgaacaattggaccaggggggagcctgcccctaaacgcaaacagagaatacacggcggcaggagctacgcatgtacccgggccctatgccagggtactgtacgtcgtcgtggaccaaaacgcagacaggtgtgtgggggtgagagtgcagggacagggtgctgtaattgacgtggatccggcgttgaattacgtgatagggggagcggatttggggatgttgccgttgatacagtggagtgtagggctgggggccgaggacatggcgcagggatcgattgcacagacgcagcgatgggtgaggatgtatggaaacgaggacgattgggaatcagcgtggcatctagtgtctagcgcgtacacagtgtacagcccggcattcaggagatcgggtgtcgcagtggagggaggattctgggcgcaaccagctgcaggggcagcaccgtttccactaggaggattggcagggtgggtgaggtacgacaatcaggcacgggcggcgcaggttgcactttgcagagagagggcggatatggcggagtgtccttggggggggtacagggagagaggggtgagaccggggagtgtggcaaactggcagtacgtaaggttcgatcccacagtggctgtaggagtagctgctcacttctggtcggtagtgaaggtgatggtggctcccgtcccagacagagcggctgctctggcggacatggcgtgggggaaggggaaggtgcaagccatgggtgaggatgtgatcaacgggcagatgggacaacctgagtccatgatgagaggggtggcgctgaacgagaaccagggactagcggcggctacagtcaggagggtggttgggctggagaacgagtcgatgcaaacaacgcactggagtacaacggaggtagcaatgaacgggtactacgggagagcaggagcaacagcacaccacgctgcatttccgttgtccgagggggggacaatgcgaaaacgaataccagctatagagatgagggagaacggggtggagggggacctgatgaacgatgatctctattcaattggaacggcagcggggtacctggcggtagaggggatggcaggtgcgcaggggggtatctgggacgtggtccagtaccagctgcctgggcctgacgatgaggcgaggggggtgatgaacacggtgggggcgatggggggatggacgagggcggtgacaccagtagacaatgtggccaccatgagggacaacggggttgagggggaaccttgtggaatagtgatgtctctaccaacaagtgggaccgctgtggtggataggttagctaatttcggattaccaccagcgagggcggaattaagagaagtaccatttggcgggtaccaaagatcagtcacaaacaccaaccacagagtcaaggtgagtgtgagtggggggcgagcagttgttcaaaaagggaacaaagccgagatgaatccagtctttgtcaataggacaccaggacaaacgaccctaggccaaccaacaacagacactacagggatgacaactgcagattttttagatatatag

SEQ ID NO: 2 - protein, 861 aa, Piscine Myocarditis Virus
MEPNTSVIATEQQQAAMREVEAEAAARDEVVEKIAFAEGAMMVQTRRLPSGKSSVGGFLGELAQNIRAMNRSLHTDTNMLTEGAMVDRARAKVHKIIREGNLDSRVFSNTGSNTMLSLWVPAVPGPPAVPEHWDVAPSWFVCRPGKKGGIKITQSASMAALNPLFRGADVGPIGTAVRADVNAFSMNAVLGALRAGGFNTEHSLVSFVEPLIRILLMGVQTQDRGTSPWDWVGGMSSRIVNPLVFTTSGNFFPGGPNLRVWGANDTVARIVNVEDYMREAAGEGRFDAGWGPEFWGGTGDDAVAVVPIRAVEAGLGEVNAGWTLAHMEYPVKVRLLDVDDRTIGPGGSLPLNANREYTAAGATHVPGPYARVLYVVVDQNADRCVGVRVQGQGAVIDVDPALNYVIGGADLGMLPLIQWSVGLGAEDMAQGSIAQTQRWVRMYGNEDDWESAWHLVSSAYTVYSPAFRRSGVAVEGGFWAQPAAGAAPFPLGGLAGWVRYDNQARAAQVALCRERADMAECPWGGYRERGVRPGSVANWQYVRFDPTVAVGVAAHFWSVVKVMVAPVPDRAAALADMAWGKGKVQAMGEDVINGQMGQPESMMRGVALNENQGLAAATVRRVVGLENESMQTTHWSTTEVAMNGYYGRAGATAHHAAFPLSEGGTMRKRIPAIEMRENGVEGDLMNDDLYSIGTAAGYLAVEGMAGAQGGIWDVVQYQLPGPDDEARGVMNTVGAMGGWTRAVTPVDNVATMRDNGVEGEPCGIVMSLPTSGTAVVDRLANFGLPPARAELREVPFGGYQRSVTNTNHRVKVSVSGGRAVVQKGNKAEMNPVFVNRTPGQTTLGQPTTDTTGMTTADFLDI